European Patent Application EP 4 406 551 A1, published July 31, 2024. Title: 無莢膜株を抗原として含むワクチン. Applicant: 国立研究開発法人　農業・食品産業技術総合研究機構. The sequence listing filed with the application follows.

SEQUENCE LISTING (2 sequences)

SEQ ID NO: 1 - DNA, 19 bp, synthetic construct
  source 1..19: mol_type = other DNA
gaaaggtctgatgctgatg

SEQ ID NO: 2 - DNA, 19 bp, synthetic construct
  source 1..19: mol_type = other DNA
tcatcccctatgcttacag